European Patent Specification EP 3 236 997 B1, published May 29, 2024. Title: DENGUE VIRUS VACCINE COMPOSITIONS AND METHODS OF USE THEREOF. Applicant: Merck Sharp & Dohme Corp. Casimiro, Danilo R. Bett, Andrew Coller, Beth-Ann Griswold Dhanasekaran, Govindarajan Chintala, Ramesh V. The sequence listing filed with the application follows.

SEQUENCE LISTING (5 sequences)

SEQ ID NO: 1 - protein, 395 aa, Dengue 1
MRCVGIGSRDFVEGLSGATWVDVVLEHGSCVTTMAKDKPTLDIELLKTEVTNPAVLRKLCIEAKISNTTTDSRCPTQGEATLVEEQDANFVCRRTFVDRGWGNGCGLFGKGSLITCAKFKCVTKLEGKIVQYENLKYSVIVTVHTGDQHQVGNESTEHGTTATITPQAPTSEIQLTDYGALTLDCSPRTGLDFNEMVLLTMKEKSWLVHKQWFLDLPLPWTSGASTSQETWNRQDLLVTFKTAHAKKQEVVVLGSQEGAMHTALTGATEIQTSGTTTIFAGHLKCRLKMDKLTLKGMSYVMCTGSFKLEKEVAETQHGTVLVQIKYEGTDAPCKIPFSTQDERGVTQNGRLITANPIVTDKEKPVNIEAEPPFGESYIVIGAGEKALKLSWFKKG

SEQ ID NO: 2 - protein, 395 aa, Dengue 2
MRCIGISNRDFVEGVSGGSWVDIVLEHGSCVTTMAKNKPTLDFELIKTEAKQPATLRKYCIEAKLTNTTTDSRCPTQGEPTLNEEQDKRFVCKHSMVDRGWGNGCGLFGKGGIVTCAMFTCKKNMEGKIVQPENLEYTVVITPHSGEEHAVGNDTGKHGKEVKITPQSSITEAELTGYGTVTMECSPRTGLDFNEMVLLQMKDKAWLVHRQWFLDLPLPWLPGADTQGSNWIQKETLVTFKNPHAKKQDVVVLGSQEGAMHTALTGATEIQMSSGNLLFTGHLKCRLRMDKLQLKGMSYSMCTGKFKVVKEIAETQHGTIVIRVQYEGDGSPCKIPFEIMDLEKRHVLGRLITVNPIVTEKDSPVNIEAEPPFGDSYIIIGVEPGQLKLDWFKKG

SEQ ID NO: 3 - protein, 393 aa, Dengue 3
MRCVGVGNRDFVEGLSGATWVDVVLEHGGCVTTMAKNKPTLDIELQKTEATQLATLRKLCIEGKITNITTDSRCPTQGEAILPEEQDQNYVCKHTYVDRGWGNGCGLFGKGSLVTCAKFQCLESIEGKVVQHENLKYTVIITVHTGDQHQVGNETQGVTAEITPQASTVEAILPEYGTLGLECSPRTGLDFNEMILLTMKNKAWMVHRQWFFDLPLPWTSGATTETPTWNRKELLVTFKNAHAKKQEVVVLGSQEGAMHTALTGATEIQNSGGTSIFAGHLKCRLKMDKLELKGMSYAMCLNTFVLKKEVSETQHGTILIKVEYKGEDAPCKIPFSTEDGQGKAHNGRLITANPVVTKKEEPVNIEAEPPFGESNIVIGIGDKALKINWYKKG

SEQ ID NO: 4 - protein, 395 aa, Dengue 4
MRCVGVGNRDFVEGVSGGAWVDLVLEHGGCVTTMAQGKPTLDFELIKTTAKEVALLRTYCIEASISNITTATRCPTQGEPYLKEEQDQQYICRRDVVDRGWGNGCGLFGKGGVVTCAKFSCSGKITGNLVQIENLEYTVVVTVHNGDTHAVGNDTSNHGVTATITPRSPSVEVKLPDYGELTLDCEPRSGIDFNEMILMKMKKKTWLVHKQWFLDLPLPWAAGADTSEVHWNYKERMVTFKVPHAKRQDVTVLGSQEGAMHSALTGATEVDSGDGNHMYAGHLKCKVRMEKLRIKGMSYTMCSGKFSIDKEMAETQHGTTVVKVKYEGAGAPCKVPIEIRDVNKEKVVGRIISSTPFAEYTNSVTNIELEPPFGDSYIVIGVGDSALTLHWFRKG

SEQ ID NO: 5 - protein, 451 aa, Artificial Sequence
  DEN4-80EZip
MRCVGVGNRDFVEGVSGGAWVDLVLEHGGCVTTMAQGKPTLDFELIKTTAKEVALLRTYCIEASISNITTATRCPTQGEPYLKEEQDQQYICRRDVVDRGWGNGCGLFGKGGVVTCAKFSCSGKITGNLVQIENLEYTVVVTVHNGDTHAVGNDTSNHGVTATITPRSPSVEVKLPDYGELTLDCEPRSGIDFNEMILMKMKKKTWLVHKQWFLDLPLPWAAGADTSEVHWNYKERMVTFKVPHAKRQDVTVLGSQEGAMHSALTGATEVDSGDGNHMYAGHLKCKVRMEKLRIKGMSYTMCSGKFSIDKEMAETQHGTTVVKVKYEGAGAPCKVPIEIRDVNKEKVVGRIISSTPFAEYTNSVTNIELEPPFGDSYIVIGVGDSALTLHWFRKGGGGSGGGGTGGGSGGGSPRMKQLEDKVEELLSKNYHLENEVARLKKLVGERGGCGG